European Patent Application EP 4 206 218 A1, published July 5, 2023. Title: PROTEINS AND BIOLOGICAL MATERIALS RELATED TO RICE (Oryza sativa L.) YIELD, AND USE THEREOF IN RICE YIELD INCREASE. Applicant: INSTITUTE OF CROP SCIENCES, CHINESE ACADEMY OF AGRICULTURAL SCIENCES. The sequence listing filed with the application follows.

SEQUENCE LISTING (21 sequences)

SEQ ID NO: 1 - protein, 214 aa, Oryza sativa L.
MEYYEQEEYATVTSAPPKRPAGRTKFRETRHPVYRGVRRRGPAGRWVCEVREPNKKSRIWLGTFATAEAAARAHDVAALALRGRGACLNFADSARLLRVDPATLATPDDIRRAAIELAESCPHDAAAAAASSSAAAVEASAAAAPAMMMQYQDDMAATPSSYDYAYYGNMDFDQPSYYYDGMGGGGEYQSWQMDGDDDGGAGGYGGGDVTLWSY

SEQ ID NO: 2 - DNA, 645 bp, Oryza sativa L.
atggagtactacgagcaggaggagtacgcgacggtgacgtcggcgccgccgaagcggccggcggggaggaccaagttcagggagacgaggcacccggtgtaccgcggcgtgcggcggcgggggcccgcggggcggtgggtgtgcgaggtcagggagcccaacaagaagtcccgcatctggctcggcaccttcgccaccgccgaggccgccgcgcgcgcccacgacgtcgccgcgctcgccctccgcggccgcggcgcgtgcctcaacttcgccgactcggcccgcctcctccgcgtcgacccggccaccctcgccacccccgacgacatccgccgcgccgccatcgagctcgccgagtcatgcccgcacgacgccgccgccgccgccgcctccagctccgccgccgccgtcgaggcctccgccgccgccgcgcccgccatgatgatgcagtaccaggacgacatggcggcgacgccgtccagctacgactacgcgtactacggcaacatggacttcgaccagccgtcctactactacgacgggatgggcggcggcggcgagtaccagagctggcagatggacggcgacgacgatggtggcgccggcggctacggcggcggcgacgtcacactctggagctactga

SEQ ID NO: 3 - DNA, 4134 bp, Oryza sativa L.
cccgtaatattgattttgattttttcttatgttgtttgaccattcgtcttaatcaagaaactttgaaattattatttattttatttatatcttactttattatccaaagtactttaagcataattttttattttttatatttgcacaaattttttgaataagaagagtggtcaaacagtgtaaaaaaagtcaaaatcacttatattatgggatggagggagtatgtgtttacctaaagtagtactctattcatattatttactaggaacaaaaaaatgccgtcgactttttattaacatttgatcaatcgtcttattcaaaatttatgtgtaaatataaaagtatttatgtcatgctttaaaaacatttgaagataaatcaagtcataataaaataaatgataaaataagacgaatggtcaagcgttgtaaagttaacggcgttatatattaaaatacgaagagagtactgcatcagtatcatactagaagaagtaataccagtactaaacagctttgatattttcgctagtagcccgcatatatcctcagttaatttgttgctttagttaaattgtgttaagagtgaattgcaccttgatctgagtatctttttttttgttatcgtagttttactttagatcacctcttaattcatggtttttactttaaaactagggaatgttacattttctagaatagatggtccaaaatgaagctctggaataaaatatagcccaatgtataattcattaataagaatagtagtataaaaatctccatgtaaaattattttcagttgattagtactcaacaaggtatattgtgtcacgtagaccataagatattgtcttgtagggatgtaagtggacaatctcactacccatataaagcctcacttgccaattactttctcaaaactttaaaagaaaaaaaattaactagaacaggtaaaagggaaaaaaaatcccgcttgtccgcttcccttggcatctggatggtcacgtggcaggaaagaacttgtacagtagtagtacgtgctagggtttgaagtaggagcgcgtgtcaatcaccaaaaaaaaaaaacaaaaaaaggcacagcagcgagtggaaaggagtcgatgggattttatgcccaaaaccgcgagagatccaccgctgtttgatgggttcgttgggacttgggaaggaatccatcggcgaatcgccgcgcggctccgatccggggcgcaagcgcaaggccaccggcccacgtactccactactcctactccgtagagaggcgacgcgtttgcgcgggcggcgccgcggccgcccaacccaaccgtcgctgcctccgtctccgtagtccgtactgcctgtgtctgcctctgctactgctgctgcctgagagcaggtaccatagcatagcaggctacaaaccagctacaaacatattttaaaaaaataaataaggagagagaatggtagcaggctacagatttatagccagctgtagcacggacttcaagacacagtgtgtatgacagatgggaccatatattaatagtgtaatatgtaactattatatgaatgagctattatattggctatagatgaatggtagttattagttggctatactattgaacttgccagagaccaaccagctactccctcacgtgcggctggattaaataaacattaatcaattaattaattatagagacaatcagttgccacttgccaattaaggaagaaggcataagtactgtagcactgcagccgcacactccacgtctccattgggaggaaatggaaaatagtttttcttttttttaaaaaaaaatagaaaatagtgctccttccgttttatattataaatcgtttgatatttttcttagtcaaaatttattaggtttgatcaaatatatagaaaaaaagaaacatgtacaacatcaaatttcattaaatttaacattgtatatattttaatataatgtttattttatattaaaaaacattactatattttgcttaaagtttgacttaaaaaaatctctactattataaaattgaagatgtttttgccggtattctagtacatcatctgtgtatgagtcggtttttaagtttgtttgcttttgaaaatatatatccgtatttgagttggtttgtaagatcgttcacttttgtatgatacaaaaggaatcatataagaaatctgtttaaaataactcacatgctaaattgagacgatcggattccaaactttagctcatgattttctaaaaatatatatatccaagtgaactcccacagtgaattttatcttaactaaactatataattaaaatagatttcacccgttgcaacgcacgatattttttctagtactccctccgtttcataatgtaagacttcaaacattggttatattcatatatgtgttaatgaatctagacacacatatatatctagattcattaacatctatatgaatatggacaatactagaaagacttacattataaaacagaggaagtaactcataaatacggaacgaaggggtagaaatatccgcatctcatacacacacagaagtggtcagccgccgcccaaaagcttgcctttgtcgccatctccacgtggccacccccatatactattgcttaacgctgtcacctcaccctctcgcggtttgagttttccacttccacggttccaccccgacacctagcgaagtactcgtagtaatccgaatcccaccgttccatccgtcgcggacgccacgctctcggctctcagctcacgtgacgtcaaccccgccaaaacgcgttattgccgtagtactacgcctcttcttccacctccatctccccctccgacatctccagccaattccagctcagctctcgccgccctcccctctcccgccacgtgcgcgccgcccctcctccaaatctccttttcttttccttttctataaataaatcaaaattcacacaccaaatcctatataaacttcttcctctccatccccttcccgctcaaactcaaacaccaacaccttcttcctcttcttcttcttccagcagcagcaacacacactactgacatggagtactacgagcaggaggagtacgcgacggtgacgtcggcgccgccgaagcggccggcggggaggaccaagttcagggagacgaggcacccggtgtaccgcggcgtgcggcggcgggggcccgcggggcggtgggtgtgcgaggtcagggagcccaacaagaagtcccgcatctggctcggcaccttcgccaccgccgaggccgccgcgcgcgcccacgacgtcgccgcgctcgccctccgcggccgcggcgcgtgcctcaacttcgccgactcggcccgcctcctccgcgtcgacccggccaccctcgccacccccgacgacatccgccgcgccgccatcgagctcgccgagtcatgcccgcacgacgccgccgccgccgccgcctccagctccgccgccgccgtcgaggcctccgccgccgccgcgcccgccatgatgatgcagtaccaggacgacatggcggcgacgccgtccagctacgactacgcgtactacggcaacatggacttcgaccagccgtcctactactacgacgggatgggcggcggcggcgagtaccagagctggcagatggacggcgacgacgatggtggcgccggcggctacggcggcggcgacgtcacactctggagctactgatgatcgcgagttggagctagcagttttgagctcaaccagctttgctcctcctatacagctaaatactgtaggagaaattaatggagattttttccttctttattttttttatattttttccaagataaaatggctgagctggtagggagttctagaaggaggaaataaagattacgagatttgtaatactactacgagggacagcatgcaaaaaagaagtataattgctatgctctctctctctctctctctcttttgtgtggagtggaataaaatgccagctctgcttatggtcagattttcacttttttttggagtgttaagacaaatgaaagctccagataaattagtgagtgctactgcttatctgaataaatgagatcattcatcatc

SEQ ID NO: 4 - DNA, 40 bp, Artificial sequence
cagtggtctcacaacatggagtactacgagcaggaggagt

SEQ ID NO: 5 - DNA, 40 bp, Artificial sequence
cagtggtctcatacatcagtagctccagagtgtgacgtcg

SEQ ID NO: 6 - DNA, 25 bp, Artificial sequence
tgtgtggcgtcgtgcgggcatgact

SEQ ID NO: 7 - DNA, 25 bp, Artificial sequence
aaacagtcatgcccgcacgacgcca

SEQ ID NO: 8 - DNA, 21 bp, Artificial sequence
catgatgatgcagtaccagga

SEQ ID NO: 9 - DNA, 22 bp, Artificial sequence
gatcatcagtagctccagagtg

SEQ ID NO: 10 - DNA, 20 bp, Artificial sequence
aagaagctgaagcatccagc

SEQ ID NO: 11 - DNA, 20 bp, Artificial sequence
ccaggacaagatgatctgcc

SEQ ID NO: 12 - DNA, 42 bp, Artificial sequence
caggtcgactctagaggatccatggagtactacgagcaggag

SEQ ID NO: 13 - DNA, 42 bp, Artificial sequence
cgatcggggaaattcgagctctcagtagctccagagtgtgac

SEQ ID NO: 14 - DNA, 25 bp, Artificial sequence
caccatggagtactacgagcaggag

SEQ ID NO: 15 - DNA, 21 bp, Artificial sequence
gtagctccagagtgtgacgtc

SEQ ID NO: 16 - DNA, 19 bp, Artificial sequence
caggaaccgcaggagtgga

SEQ ID NO: 17 - DNA, 20 bp, Artificial sequence
ccagaaacccacgtcatgcc

SEQ ID NO: 18 - DNA, 21 bp, Artificial sequence
catgatgatgcagtaccagga

SEQ ID NO: 19 - DNA, 22 bp, Artificial sequence
gatcatcagtagctccagagtg

SEQ ID NO: 20 - DNA, 22 bp, Artificial sequence
gcaccacctgaaaggaagtaca

SEQ ID NO: 21 - DNA, 22 bp, Artificial sequence
cgattcctggacctgcctcatc